European Patent Application EP 4 296 281 A1, published December 27, 2023. Title: Targeting modules against CD123 for use in a method for stimulating a chimeric antigen receptor-mediated immune response in a mammal. Applicant: AvenCell Therapeutics Inc. The sequence listing filed with the application follows.

SEQUENCE LISTING (32 sequences)

SEQ ID NO: 1 - DNA, 1575 bp, Artificial Sequence
  targeting module
gaagtgcagctgcagcagtctggccccgagctggtcaaaccaggcgccagcgtgaagatgagctgcaaggccagcggctacaccttcaccgactactacatgaagtgggtcaagcagagccacggcaagagcctggaatggatcggcgacatcatccccagcaacggcgccaccttctacaaccagaagttcaagggcaaggccaccctgaccgtggacagaagcagcagcaccgcctacatgcacctgaacagcctgaccagcgaggacagcgccgtgtactactgcaccagaagccatctgctgcgggccagttggttcgcttattggggccagggcaccctggtcacagtgtctgccgcctctggaggaggaggtagtggcggaggtgggtccggtggcggtggctctgacttcgtgatgacccagagccctagcagcctgaccgtgacagccggcgagaaagtgaccatgagctgcaagagcagccagagcctgctgaactccggcaaccagaagaactacctgacctggtatctgcagaagcccggacagccccccaagctgctgatctactgggccagcaccagagaaagcggcgtgcccgatagattcacaggcagcggcagcggcaccgacttcaccctgacaatcagcagcgtgcaggccgaggacctggccgtgtactattgccagaacgactacagctacccctacaccttcggaggcgggaccaagctggaaatcaaggcggccgctcgaggacaagtgcaactggtccagtcaggtgctgaggtgaaaaaacccggagccagtgtcaaagtaagctgcaaggcctctgggtatactttcacccattactatatatactgggttcgtcaagctccaggtcaggggcttgagtggatgggtggagtcaacccttcgaacggtggcactcacttcaatgaaaagtttaaaagccgcgtaaccatgacgcgagatacttccatttccacagcttatatggaacttagtaggttacgcagtgatgacacggccgtttattactgtgctagaagtgaatatgattatgggttgggtttcgcttactggggccagggaaccctcgtcaccgtgtccagtggtggtggaggatccggtggtggcggttctggcggaggcggatccgacattgttatgacgcagagccctgattcactcgcagtgtccctaggagagcgggccaccatcaactgtaaaagttctcagtccctgctgaacagcaggacgcctaagaattacctggcatggtaccaacagaaacctggacagccgcctaagctgctcatttactgggcctccacacggaagagcggcgtgcccgaccggttttccgggagcggctccggcaccgactttaccttgaccatcagttccctgcaggcagaagacgtggccgtatactattgcaagcaatcttacaatctcctgacatttggcggcggcacaaaagtggagatcaaagggcccgaacaaaaactcatctcagaagaggatctgaatagcgccgtcgaccatcatcatcatcatcat

SEQ ID NO: 2 - protein, 525 aa, Artificial Sequence
  targeting module
EVQLQQSGPELVKPGASVKMSCKASGYTFTDYYMKWVKQSHGKSLEWIGDIIPSNGATFYNQKFKGKATLTVDRSSSTAYMHLNSLTSEDSAVYYCTRSHLLRASWFAYWGQGTLVTVSAASGGGGSGGGGSGGGGSDFVMTQSPSSLTVTAGEKVTMSCKSSQSLLNSGNQKNYLTWYLQKPGQPPKLLIYWASTRESGVPDRFTGSGSGTDFTLTISSVQAEDLAVYYCQNDYSYPYTFGGGTKLEIKAAARGQVQLVQSGAEVKKPGASVKVSCKASGYTFTHYYIYWVRQAPGQGLEWMGGVNPSNGGTHFNEKFKSRVTMTRDTSISTAYMELSRLRSDDTAVYYCARSEYDYGLGFAYWGQGTLVTVSSGGGGSGGGGSGGGGSDIVMTQSPDSLAVSLGERATINCKSSQSLLNSRTPKNYLAWYQQKPGQPPKLLIYWASTRKSGVPDRFSGSGSGTDFTLTISSLQAEDVAVYYCKQSYNLLTFGGGTKVEIKGPEQKLISEEDLNSAVDHHHHHH

SEQ ID NO: 3 - protein, 526 aa, Artificial Sequence
  targeting module
GQVQLVQSGAEVKKPGSSVKVSCKASGYTFTDYYIHWVRQAPGQGLEWMGDIIPSNGATFYNQRFKGRVTITADESTSTAYMELSSLRSEDTAVYYCTRSHLLRASWFAYWGQGTLVTVSSASGGGGSGGGGSGGGGSDIVMTQTPLSLSVTPGQPASISCRSSQSLLNSGNQKNYLTWYLQKPGQSPQLLIYWASTRFIGVPDRFSGSGSGTDFTLKISRVEAEDVGVYYCQNDYSYPYTFGQGTKLEIKAAARGDIVMTQSPDSLAVSLGERATINCKSSQSLLNSRTPKNYLAWYQQKPGQPPKLLIYWASTRKSGVPDRFSGSGSGTDFTLTISSLQAEDVAVYYCKQSYNLLTFGGGTKVEIKGGGGSGGGGSGASAAGGGGSGGGGSQVQLVQSGAEVKKPGASVKVSCKASGYTFTHYYIYWVRQAPGQGLEWMGGVNPSNGGTHFNEKFKSRVTMTRDTSISTAYMELSRLRSDDTAVYYCARSEYDYGLGFAYWGQGTLVTVSSGGGGSHHHHHHHH

SEQ ID NO: 4 - protein, 526 aa, Artificial Sequence
  targeting module
GQVQLVQSGAEVKKPGASVKMSCKASGYTFTDYYMKWVKQAPGQGLEWIGDIIPSNGATFYNQKFQGRATLTVDTSTSTAYMELSSLRSEDTAVYYCTRSHLLRASWFAYWGQGTLVTVSSASGGGGSGGGGSGGGGSDIVMTQSPDSLAVSLGERATINCKSSQSLLNSGNQKNYLTWYLQKPGQPPKLLIYWASTRESGVPDRFSGSGSGTDFTLTISSVQAEDVAVYYCQNDYSYPYTFGGGTKLEIKAAARGDIVMTQSPDSLAVSLGERVTMNCKSSQSLLNSRTPKNYLAWYQQKPGQSPKLLIYWASTRKSGVPDRFSGSGSGTDFTLTISSVQAEDVAVYYCKQSYNLLTFGGGTKLEIKGGGGSGGGGSGASAAGGGGSGGGGSQVQLVESGAEVVKPGASVKLSCKASGYAFTHYYIYWIKQAPGQGLEWIGGVNPSNGGTHFNEKFKSRATLTVDTSISTAYMELSRLRSDDTAVYYCTRSEYDYGLGFAYWGQGTLVTVSSGGGGSHHHHHHHH

SEQ ID NO: 5 - protein, 525 aa, Artificial Sequence
  targeting module
EVQLQQSGPELVKPGASVKMSCKASGYTFTDYYMKWVKQSHGKSLEWIGDIIPSNGATFYNQKFKGKATLTVDRSSSTAYMHLNSLTSEDSAVYYCTRSHLLRASWFAYWGQGTLVTVSAASGGGGSGGGGSGGGGSDFVMTQSPSSLTVTAGEKVTMSCKSSQSLLNSGNQKNYLTWYLQKPGQPPKLLIYWASTRESGVPDRFTGSGSGTDFTLTISSVQAEDLAVYYCQNDYSYPYTFGGGTKLEIKAAARGDIVMTQSPDSLAVSLGERATINCKSSQSLLNSRTPKNYLAWYQQKPGQPPKLLIYWASTRKSGVPDRFSGSGSGTDFTLTISSLQAEDVAVYYCKQSYNLLTFGGGTKVEIKGGGGSGGGGSGASAAGGGGSGGGGSQVQLVQSGAEVKKPGASVKVSCKASGYTFTHYYIYWVRQAPGQGLEWMGGVNPSNGGTHFNEKFKSRVTMTRDTSISTAYMELSRLRSDDTAVYYCARSEYDYGLGFAYWGQGTLVTVSSGGGGSHHHHHHHH

SEQ ID NO: 6 - protein, 525 aa, Artificial Sequence
  targeting module
EVQLQQSGPELVKPGASVKMSCKASGYTFTDYYMKWVKQSHGKSLEWIGDIIPSNGATFYNQKFKGKATLTVDRSSSTAYMHLNSLTSEDSAVYYCTRSHLLRASWFAYWGQGTLVTVSAASGGGGSGGGGSGGGGSDFVMTQSPSSLTVTAGEKVTMSCKSSQSLLNSGNQKNYLTWYLQKPGQPPKLLIYWASTRESGVPDRFTGSGSGTDFTLTISSVQAEDLAVYYCQNDYSYPYTFGGGTKLEIKAAARGDIVMTQSPDSLAVSLGERVTMNCKSSQSLLNSRTPKNYLAWYQQKPGQSPKLLIYWASTRKSGVPDRFSGSGSGTDFTLTISSVQAEDVAVYYCKQSYNLLTFGGGTKLEIKGGGGSGGGGSGASAAGGGGSGGGGSQVQLVESGAEVVKPGASVKLSCKASGYAFTHYYIYWIKQAPGQGLEWIGGVNPSNGGTHFNEKFKSRATLTVDTSISTAYMELSRLRSDDTAVYYCTRSEYDYGLGFAYWGQGTLVTVSSGGGGSHHHHHHHH

SEQ ID NO: 7 - protein, 526 aa, Artificial Sequence
  targeting module
GQVQLVQSGAEVKKPGASVKMSCKASGYTFTDYYMKWVKQAPGQGLEWIGDIIPSNGATFYNQKFQGRATLTVDTSTSTAYMELSSLRSEDTAVYYCTRSHLLRASWFAYWGQGTLVTVSSASGGGGSGGGGSGGGGSDIVMTQSPDSLAVSLGERATINCKSSQSLLNSGNQKNYLTWYLQKPGQPPKLLIYWASTRESGVPDRFSGSGSGTDFTLTISSVQAEDVAVYYCQNDYSYPYTFGGGTKLEIKAAARGDIVMTQSPDSLAVSLGERATINCKSSQSLLNSRTPKNYLAWYQQKPGQPPKLLIYWASTRKSGVPDRFSGSGSGTDFTLTISSLQAEDVAVYYCKQSYNLLTFGGGTKVEIKGGGGSGGGGSGASAAGGGGSGGGGSQVQLVQSGAEVKKPGASVKVSCKASGYTFTHYYIYWVRQAPGQGLEWMGGVNPSNGGTHFNEKFKSRVTMTRDTSISTAYMELSRLRSDDTAVYYCARSEYDYGLGFAYWGQGTLVTVSSGGGGSHHHHHHHH

SEQ ID NO: 8 - protein, 526 aa, Artificial Sequence
  targeting module
GQVQLVQSGAEVKKPGASVKMSCKASGYTFTDYYMKWVKQAPGQGLEWIGDIIPSNGATFYNQKFKGRATLTVDKSTSTAYMELSSLRSEDTAVYYCTRSHLLRASWFAYWGQGTLVTVSSASGGGGSGGGGSGGGGSDFVMTQSPDSLAVSLGERATMNCKSSQSLLNSGNQKNYLTWYLQKPGQPPKLLIYWASTRESGVPDRFSGSGSGTDFTLTISSVQAEDVAVYYCQNDYSYPYTFGGGTKLEIKAAARGDIVMTQSPDSLAVSLGERATINCKSSQSLLNSRTPKNYLAWYQQKPGQPPKLLIYWASTRKSGVPDRFSGSGSGTDFTLTISSLQAEDVAVYYCKQSYNLLTFGGGTKVEIKGGGGSGGGGSGASAAGGGGSGGGGSQVQLVQSGAEVKKPGASVKVSCKASGYTFTHYYIYWVRQAPGQGLEWMGGVNPSNGGTHFNEKFKSRVTMTRDTSISTAYMELSRLRSDDTAVYYCARSEYDYGLGFAYWGQGTLVTVSSGGGGSHHHHHHHH

SEQ ID NO: 9 - protein, 525 aa, Artificial Sequence
  targeting module
EVQLVQSGAEVKKPGASVKMSCKASGYTFTDYYMKWVKQAPGQGLEWIGDIIPSNGATFYNQKFKGRATLTVDRSTSTAYMELSSLRSEDTAVYYCTRSHLLRASWFAYWGQGTLVTVSSASGGGGSGGGGSGGGGSDFVMTQSPDSLAVSLGERATINCESSQSLLNTGNQKNYLTWYLQKPGQPPKLLIYWASTRESGVPDRFSGSGSGTDFTLTISSVQAEDVAVYYCQNDYSYPYTFGGGTKLEIKAAARGDIVMTQSPDSLAVSLGERATINCKSSQSLLNSRTPKNYLAWYQQKPGQPPKLLIYWASTRKSGVPDRFSGSGSGTDFTLTISSLQAEDVAVYYCKQSYNLLTFGGGTKVEIKGGGGSGGGGSGASAAGGGGSGGGGSQVQLVQSGAEVKKPGASVKVSCKASGYTFTHYYIYWVRQAPGQGLEWMGGVNPSNGGTHFNEKFKSRVTMTRDTSISTAYMELSRLRSDDTAVYYCARSEYDYGLGFAYWGQGTLVTVSSGGGGSHHHHHHHH

SEQ ID NO: 10 - protein, 525 aa, Artificial Sequence
  targeting module
EVQLVQSGAEVKKPGASVKMSCKASGYTFTDYYMKWVKQAPGQGLEWIGDIIPSNGATFYNQKFKGRATLTVDRSTSTAYMELSSLRSEDTAVYYCTRSHLLRASWFAYWGQGTLVTVSSASGGGGSGGGGSGGGGSDFVMTQSPDSLAVSLGERATINCESSQSLLNTGNQKNYLTWYLQKPGQPPKLLIYWASTRESGVPDRFSGSGSGTDFTLTISSVQAEDVAVYYCQNDYSYPYTFGGGTKLEIKAAARGDIVMTQSPDSLAVSLGERVTMNCKSSQSLLNSRTPKNYLAWYQQKPGQSPKLLIYWASTRKSGVPDRFSGSGSGTDFTLTISSVQAEDVAVYYCKQSYNLLTFGGGTKLEIKGGGGSGGGGSGASAAGGGGSGGGGSQVQLVESGAEVVKPGASVKLSCKASGYAFTHYYIYWIKQAPGQGLEWIGGVNPSNGGTHFNEKFKSRATLTVDTSISTAYMELSRLRSDDTAVYYCTRSEYDYGLGFAYWGQGTLVTVSSGGGGSHHHHHHHH

SEQ ID NO: 11 - DNA, 1578 bp, Artificial Sequence
  targeting module
ggacaggtgcagctggtgcagtctggcgccgaagtgaagaaacctggctcctccgtgaaggtgtcctgcaaggcttctggctacacctttaccgactactacatccactgggtccgacaggcccctggacaaggattggagtggatgggcgacatcatcccttctaacggcgccaccttctacaaccagcggttcaagggcagagtgaccatcaccgccgacgagtctacctccaccgcctacatggaactgtccagcctgagatctgaggacaccgccgtgtactactgtaccagatctcatctgctgcgggccagttggttcgcttattggggacagggcaccctggtcaccgtgtcatctgcatctggtggcggaggatctggcggaggtggaagcggcggaggcggatctgatatcgtgatgacccagacacctctgagcctgagcgtgacacctggacagcctgcctccatctcctgcagatcctctcagtccctgctgaactccggcaaccagaagaactacctgacctggtatctgcagaagcccggccagtctcctcagctgctgatctactgggcctccaccagattcatcggcgtgcccgatagattctccggctctggatctggcaccgacttcaccctgaagatctccagagtggaagccgaggacgtgggcgtgtactattgccagaacgactacagctacccctacaccttcggccagggcaccaagctggaaatcaaggctgccgctcgaggagacattgtgatgacacagagccccgacagcctggctgtgtctctgggagagagagccaccatcaactgcaagtccagccagagcctgctgaattctcggacccctaagaattacctcgcttggtatcagcaaaagcctgggcagccaccaaagctgctcatctattgggcttctacccggaagtccggcgtgccagacaggtttagcggatctggctccggcacagactttacactgaccatcagctccctgcaggccgaggatgtggctgtgtattactgcaagcagtcctacaacctgctgaccttcggaggcggcaccaaggtcgagatcaaaggtggtggtggtagtggcggtggtggatcaggcgcttctgctgctggcggtggcggttctggcggcggtggttctcaagttcagctggttcagagcggagctgaagtgaaaaagccaggcgccagcgtgaaagtgtcttgtaaagcctccggctacacattcacccactattatatctattgggtccgccaggctccaggccagggacttgaatggatgggaggcgtgaacccttccaatggcggcacccacttcaacgagaagttcaagtctcgcgtgaccatgaccagggacaccagcatcagcaccgcttatatggaattgagccggctgcggagcgacgatacagccgtgtattattgcgccagaagcgagtacgactacggcctgggctttgcttactggggccagggaacactcgtgacagtttctagtggtggcggcggaagccaccaccatcatcaccatcaccac

SEQ ID NO: 12 - DNA, 1578 bp, Artificial Sequence
  targeting module
ggacaggtgcagctggtgcagtctggcgccgaagtgaaaaagcctggcgcctccgtgaagatgtcctgcaaggcttctggctacaccttcaccgactactacatgaaatgggtcaagcaggcccctggacagggccttgagtggatcggagacatcatcccttctaacggcgccaccttctacaaccagaagttccagggcagagctaccctgaccgtggacacctctacctccaccgcctacatggaactgtccagcctgagatctgaggacaccgccgtgtactactgtaccagatctcatctgctgcgggccagttggttcgcttattggggacagggcaccctggtcaccgtgtcatctgcatctggtggcggaggatctggcggaggtggaagcggcggaggcggatctgatatcgtgatgacccagtctcctgacagcctggctgtgtctctgggcgagagagccaccatcaactgcaagtcctctcagtccctgctgaactccggcaatcagaagaactacctgacctggtatctgcagaagcccggccagcctcctaagctgctgatctactgggcctccaccagagaatctggcgtgcccgatagattctccggctctggatctggcaccgactttaccctgacaatctccagcgtgcaggccgaggatgtggctgtgtactattgccagaacgactacagctacccttacaccttcggaggcggcaccaagctggaaatcaaggctgcagctcgaggagacattgtgatgacacagagccccgatagtctggcagtgtccctcggagaacgcgtgaccatgaactgtaaatccagccagagcctgctgaattctcggacccctaagaattacctcgcttggtatcaacagaagcctgggcagagccccaaactgctcatctattgggcttctacccggaagtccggcgtgccagacagattttctggcagcggctccggcacagactttacactcaccatcagctccgtgcaagctgaggacgtggccgtctattactgcaagcagtcctacaacctgctgacctttggcggcggaacaaagctcgagatcaaaggcggtggtggttcaggtggtggtggaagtggtgcttctgctgctggcggtggcggttctggcggcggtggttctcaagttcagctggtggaatccggcgctgaggttgtgaaacctggcgcaagcgtgaagctgagctgcaaggcaagcggctacgcttttacccactactatatctactggattaagcaggctcccggccagggactcgaatggattggcggagtgaacccttccaatggcggcacccacttcaacgagaagttcaagtctcgggccacactgacagtggatacctccatcagcaccgcttatatggaattgagccggctgcggagcgacgataccgctgtctactactgcacaagaagcgagtacgactacggcctgggctttgcttactggggccagggaacactcgtgacagtttctagtggcggcggaggaagccaccaccatcaccatcatcaccac

SEQ ID NO: 13 - DNA, 1575 bp, Artificial Sequence
  targeting module
gaggtccagctgcagcagtctggccctgagcttgtgaaacctggcgcctccgtgaagatgtcctgcaaggcttctggctacaccttcaccgactactacatgaaatgggtcaagcagtcccacggcaagtccctggaatggatcggcgacatcatcccttctaacggcgccaccttctacaaccagaagttcaagggcaaagctaccctgaccgtggacagatcctcctccaccgcttacatgcacctgaactccctgacctccgaggactccgccgtgtactactgcaccagatctcatctgctgcgggccagttggttcgcttattggggacagggcaccctggtcaccgtgtctgctgcatctggcggaggtggaagcggaggcggaggttctggcggtggcggatctgatttcgtgatgacccagtctccttcctctctgaccgtgaccgctggcgagaaagtgaccatgagctgcaagtcctctcagtccctgctgaactccggcaatcagaagaattacctgacctggtatctgcagaagcccggccagcctcctaagctgctgatctactgggcctccaccagagaatctggcgtgcccgatagattcaccggctctggatctggcaccgactttaccctgacaatctccagcgtgcaggccgaggatctggctgtgtactattgccagaacgactacagctacccttacaccttcggcggaggcaccaagctggaaatcaaggctgcagctcgaggagacattgtgatgacacagagccccgacagcctggctgtgtctctgggagagagagccaccatcaactgcaagtccagccagagcctgctgaattctcggacccctaagaattacctcgcttggtatcagcaaaagcctgggcagccaccaaagctgctcatctattgggcttctacccggaagtccggcgtgccagacaggtttagcggatctggctccggcacagactttacactgaccatcagctccctgcaggccgaggatgtggctgtgtattactgcaagcagtcctacaacctgctgaccttcggaggcggcaccaaggtcgagatcaaaggtggtggtggtagtggcggtggtggatcaggcgcttctgctgctggcggtggcggttctggcggcggtggttctcaagttcagctggttcagagcggagctgaagtgaaaaagccaggcgccagcgtgaaagtgtcttgtaaagcctccggctacacattcacccactattatatctattgggtccgccaggctccaggccagggacttgaatggatgggaggcgtgaacccttccaatggcggcacccacttcaacgagaagttcaagtctcgcgtgaccatgaccagggacaccagcatcagcaccgcttatatggaattgagccggctgcggagcgacgatacagccgtgtattattgcgccagaagcgagtacgactacggcctgggctttgcttactggggccagggaacactcgtgacagtttctagtggtggcggcggaagccaccaccatcatcaccatcaccac

SEQ ID NO: 14 - DNA, 1575 bp, Artificial Sequence
  targeting module
gaggtccagctgcagcagtctggccctgagcttgtgaaacctggcgcctccgtgaagatgtcctgcaaggcttctggctacaccttcaccgactactacatgaaatgggtcaagcagtcccacggcaagtccctggaatggatcggcgacatcatcccttctaacggcgccaccttctacaaccagaagttcaagggcaaagctaccctgaccgtggacagatcctcctccaccgcttacatgcacctgaactccctgacctccgaggactccgccgtgtactactgcaccagatctcatctgctgcgggccagttggttcgcttattggggacagggcaccctggtcaccgtgtctgctgcatctggcggaggtggaagcggaggcggaggttctggcggtggcggatctgatttcgtgatgacccagtctccttcctctctgaccgtgaccgctggcgagaaagtgaccatgagctgcaagtcctctcagtccctgctgaactccggcaatcagaagaattacctgacctggtatctgcagaagcccggccagcctcctaagctgctgatctactgggcctccaccagagaatctggcgtgcccgatagattcaccggctctggatctggcaccgactttaccctgacaatctccagcgtgcaggccgaggatctggctgtgtactattgccagaacgactacagctacccttacaccttcggcggaggcaccaagctggaaatcaaggctgcagctcgaggagacattgtgatgacacagagccccgatagtctggcagtgtccctcggagaacgcgtgaccatgaactgtaaatccagccagagcctgctgaattctcggacccctaagaattacctcgcttggtatcaacagaagcctgggcagagccccaaactgctcatctattgggcttctacccggaagtccggcgtgccagacagattttctggcagcggctccggcacagactttacactcaccatcagctccgtgcaagctgaggacgtggccgtctattactgcaagcagtcctacaacctgctgacctttggcggcggaacaaagctcgagatcaaaggcggtggtggttcaggtggtggtggaagtggtgcttctgctgctggcggtggcggttctggcggcggtggttctcaagttcagctggtggaatccggcgctgaggttgtgaaacctggcgcaagcgtgaagctgagctgcaaggcaagcggctacgcttttacccactactatatctactggattaagcaggctcccggccagggactcgaatggattggcggagtgaacccttccaatggcggcacccacttcaacgagaagttcaagtctcgggccacactgacagtggatacctccatcagcaccgcttatatggaattgagccggctgcggagcgacgataccgctgtctactactgcacaagaagcgagtacgactacggcctgggctttgcttactggggccagggaacactcgtgacagtttctagtggcggcggaggaagccaccaccatcaccatcatcaccac

SEQ ID NO: 15 - DNA, 1578 bp, Artificial Sequence
  targeting module
ggacaggtgcagctggtgcagtctggcgccgaagtgaaaaagcctggcgcctccgtgaagatgtcctgcaaggcttctggctacaccttcaccgactactacatgaaatgggtcaagcaggcccctggacagggccttgagtggatcggagacatcatcccttctaacggcgccaccttctacaaccagaagttccagggcagagctaccctgaccgtggacacctctacctccaccgcctacatggaactgtccagcctgagatctgaggacaccgccgtgtactactgtaccagatctcatctgctgcgggccagttggttcgcttattggggacagggcaccctggtcaccgtgtcatctgcatctggtggcggaggatctggcggaggtggaagcggcggaggcggatctgatatcgtgatgacccagtctcctgacagcctggctgtgtctctgggcgagagagccaccatcaactgcaagtcctctcagtccctgctgaactccggcaatcagaagaactacctgacctggtatctgcagaagcccggccagcctcctaagctgctgatctactgggcctccaccagagaatctggcgtgcccgatagattctccggctctggatctggcaccgactttaccctgacaatctccagcgtgcaggccgaggatgtggctgtgtactattgccagaacgactacagctacccttacaccttcggaggcggcaccaagctggaaatcaaggctgcagctcgaggagacattgtgatgacacagagccccgacagcctggctgtgtctctgggagagagagccaccatcaactgcaagtccagccagagcctgctgaattctcggacccctaagaattacctcgcttggtatcagcaaaagcctgggcagccaccaaagctgctcatctattgggcttctacccggaagtccggcgtgccagacaggtttagcggatctggctccggcacagactttacactgaccatcagctccctgcaggccgaggatgtggctgtgtattactgcaagcagtcctacaacctgctgaccttcggaggcggcaccaaggtcgagatcaaaggtggtggtggtagtggcggtggtggatcaggcgcttctgctgctggcggtggcggttctggcggcggtggttctcaagttcagctggttcagagcggagctgaagtgaaaaagccaggcgccagcgtgaaagtgtcttgtaaagcctccggctacacattcacccactattatatctattgggtccgccaggctccaggccagggacttgaatggatgggaggcgtgaacccttccaatggcggcacccacttcaacgagaagttcaagtctcgcgtgaccatgaccagggacaccagcatcagcaccgcttatatggaattgagccggctgcggagcgacgatacagccgtgtattattgcgccagaagcgagtacgactacggcctgggctttgcttactggggccagggaacactcgtgacagtttctagtggtggcggcggaagccaccaccatcatcaccatcaccac

SEQ ID NO: 16 - DNA, 1578 bp, Artificial Sequence
  targeting module
ggacaggtgcagctggtgcagtctggcgccgaagttaagaaacctggcgcctccgtgaagatgtcctgcaaggcttctggctacaccttcaccgactactacatgaaatgggtcaagcaggcccctggacagggccttgagtggatcggagacatcatcccttctaacggcgccaccttctacaaccagaagttcaagggcagagctaccctgaccgtggacaagtctacctccaccgcctacatggaactgtccagcctgagatctgaggacaccgccgtgtactactgtaccagatctcatctgctgcgggccagttggttcgcttattggggacagggcacactggtcaccgtgtcctctgcatctggtggcggaggatctggcggaggtggaagcggcggaggcggatctgatttcgtgatgacccagtctcctgacagcctggctgtgtctctcggcgagagggctaccatgaactgcaagtcctctcagtccctgctgaactccggcaatcagaagaactacctgacctggtatctgcagaagcccggccagcctcctaagctgctgatctactgggcctccaccagagaatctggcgtgcccgatagattctccggctctggctctggcaccgactttaccctgacaatcagctccgtgcaggccgaggatgtggctgtgtactattgccagaacgactacagctacccttacaccttcggaggcggcaccaagctggaaatcaaagcggccgctcgaggagacattgtgatgacacagagccccgacagcctggctgtgtctctgggagagagagccaccatcaactgcaagtccagccagagcctgctgaattctcggacccctaagaattacctcgcttggtatcagcaaaagcctgggcagccaccaaagctgctcatctattgggcttctacccggaagtccggcgtgccagacaggtttagcggatctggctccggcacagactttacactgaccatcagctccctgcaggccgaggatgtggctgtgtattactgcaagcagtcctacaacctgctgaccttcggaggcggcaccaaggtcgagatcaaaggtggtggtggtagtggcggtggtggatcaggcgcttctgctgctggcggtggcggttctggcggcggtggttctcaagttcagctggttcagagcggagctgaagtgaaaaagccaggcgccagcgtgaaagtgtcttgtaaagcctccggctacacattcacccactattatatctattgggtccgccaggctccaggccagggacttgaatggatgggaggcgtgaacccttccaatggcggcacccacttcaacgagaagttcaagtctcgcgtgaccatgaccagggacaccagcatcagcaccgcttatatggaattgagccggctgcggagcgacgatacagccgtgtattattgcgccagaagcgagtacgactacggcctgggctttgcttactggggccagggaacactcgtgacagtttctagtggtggcggcggaagccaccaccatcatcaccatcaccac

SEQ ID NO: 17 - DNA, 1575 bp, Artificial Sequence
  targeting module
gaagtgcagctggtgcagtctggcgccgaagtgaagaaacctggcgcctccgtgaagatgtcctgcaaggcttctggctacaccttcaccgactactacatgaaatgggtcaagcaggcccctggacagggccttgagtggatcggagacatcatcccttctaacggcgccaccttctacaaccagaagttcaagggcagagctaccctgaccgtggacagatctacctccaccgcctacatggaactgtccagcctgagatctgaggacaccgccgtgtactactgtaccagatctcatctgctgcgggccagttggttcgcttattggggacagggcaccctggtcaccgtgtcatctgcatctggtggcggaggatctggcggaggtggaagcggcggaggcggatctgatttcgtgatgacccagtctcctgacagcctggctgtgtctctgggcgagagagccaccatcaactgcgagtcctctcagtccctgctgaacaccggcaatcagaagaactacctgacctggtatctgcagaagcccggccagcctcctaagctgctgatctactgggcctccaccagagaatctggcgtgcccgatagattctccggctctggatctggcaccgactttaccctgacaatctccagcgtgcaggccgaggatgtggctgtgtactattgccagaacgactacagctacccttacaccttcggaggcggcaccaagctggaaatcaaagcggccgctcgaggagacattgtgatgacacagagccccgacagcctggctgtgtctctgggagagagagccaccatcaactgcaagtccagccagagcctgctgaattctcggacccctaagaattacctcgcttggtatcagcaaaagcctgggcagccaccaaagctgctcatctattgggcttctacccggaagtccggcgtgccagacaggtttagcggatctggctccggcacagactttacactgaccatcagctccctgcaggccgaggatgtggctgtgtattactgcaagcagtcctacaacctgctgaccttcggaggcggcaccaaggtcgagatcaaaggtggtggtggtagtggcggtggtggatcaggcgcttctgctgctggcggtggcggttctggcggcggtggttctcaagttcagctggttcagagcggagctgaagtgaaaaagccaggcgccagcgtgaaagtgtcttgtaaagcctccggctacacattcacccactattatatctattgggtccgccaggctccaggccagggacttgaatggatgggaggcgtgaacccttccaatggcggcacccacttcaacgagaagttcaagtctcgcgtgaccatgaccagggacaccagcatcagcaccgcttatatggaattgagccggctgcggagcgacgatacagccgtgtattattgcgccagaagcgagtacgactacggcctgggctttgcttactggggccagggaacactcgtgacagtttctagtggtggcggcggaagccaccaccatcatcaccatcaccac

SEQ ID NO: 18 - DNA, 1575 bp, Artificial Sequence
  targeting module
gaagtgcagctggtgcagtctggcgccgaagtgaagaaacctggcgcctccgtgaagatgtcctgcaaggcttctggctacaccttcaccgactactacatgaaatgggtcaagcaggcccctggacagggccttgagtggatcggagacatcatcccttctaacggcgccaccttctacaaccagaagttcaagggcagagctaccctgaccgtggacagatctacctccaccgcctacatggaactgtccagcctgagatctgaggacaccgccgtgtactactgtaccagatctcatctgctgcgggccagttggttcgcttattggggacagggcaccctggtcaccgtgtcatctgcatctggtggcggaggatctggcggaggtggaagcggcggaggcggatctgatttcgtgatgacccagtctcctgacagcctggctgtgtctctgggcgagagagccaccatcaactgcgagtcctctcagtccctgctgaacaccggcaatcagaagaactacctgacctggtatctgcagaagcccggccagcctcctaagctgctgatctactgggcctccaccagagaatctggcgtgcccgatagattctccggctctggatctggcaccgactttaccctgacaatctccagcgtgcaggccgaggatgtggctgtgtactattgccagaacgactacagctacccttacaccttcggaggcggcaccaagctggaaatcaaagcggccgctcgaggagacattgtgatgacacagagccccgatagtctggcagtgtccctcggagaacgcgtgaccatgaactgtaaatccagccagagcctgctgaattctcggacccctaagaattacctcgcttggtatcaacagaagcctgggcagagccccaaactgctcatctattgggcttctacccggaagtccggcgtgccagacagattttctggcagcggctccggcacagactttacactcaccatcagctccgtgcaagctgaggacgtggccgtctattactgcaagcagtcctacaacctgctgacctttggcggcggaacaaagctcgagatcaaaggcggtggtggttcaggtggtggtggaagtggtgcttctgctgctggcggtggcggttctggcggcggtggttctcaagttcagctggtggaatccggcgctgaggttgtgaaacctggcgcaagcgtgaagctgagctgcaaggcaagcggctacgcttttacccactactatatctactggattaagcaggctcccggccagggactcgaatggattggcggagtgaacccttccaatggcggcacccacttcaacgagaagttcaagtctcgggccacactgacagtggatacctccatcagcaccgcttatatggaattgagccggctgcggagcgacgataccgctgtctactactgcacaagaagcgagtacgactacggcctgggctttgcttactggggccagggaacactcgtgacagtttctagtggcggcggaggaagccaccaccatcaccatcatcaccac

SEQ ID NO: 19 - protein, 113 aa, Artificial Sequence
  Humanized scFv VL chain
  MISC_FEATURE (24)..(24): Xaa can be any naturally occurring amino acid
  MISC_FEATURE (35)..(35): Xaa can be any naturally occurring amino acid
  MISC_FEATURE (61)..(61): Xaa can be any naturally occurring amino acid
  MISC_FEATURE (101)..(101): Xaa can be any naturally occurring amino acid
DIVMTQSPDSLAVSLGERATINCXSSQSLLNSRTXKNYLAWYQQKPGQPPKLLIYWASTRXSGVPDRFSGSGSGTDFTLTISSLQAEDVAVYYCKQSYNLXTFGGGTKVEILK

SEQ ID NO: 20 - protein, 120 aa, Artificial Sequence
  Humanized scFv VH chain
QVQLVQSGAEVKKPGASVKVSCKASGYTFTHYYIYWVRQAPGQGLEWMGGVNPSNGGTHFNEKFKSRVTMTRDTSISTAYMELSRLRSDDTAVYYCARSEYDYGLGFAYWGQGTLVTVSS

SEQ ID NO: 21 - protein, 112 aa, Artificial Sequence
  Humanized scFv VL chain
DIVMTQSPDSLAVSLGERATINCKSSQSLLNSRTPKNYLAWYQQKPGQPPKLLIYWASTRKSGVPDRFSGSGSGTDFTLTISSLQAEDVAVYYCKQSYNLLTFGGGTKVEIK

SEQ ID NO: 22 - protein, 119 aa, Mus musculus
EVQLQQSGPELVKPGASVKMSCKASGYTFTDYYMKWVKQSHGKSLEWIGDIIPSNGATFYNQKFKGKATLTVDRSSSTAYMHLNSLTSEDSAVYYCTRSHLLRASWFAYWGQGTLVTVS

SEQ ID NO: 23 - protein, 113 aa, Mus musculus
DFVMTQSPSSLTVTAGEKVTMSCKSSQSLLNSGNQKNYLTWYLQKPGQPPKLLIYWASTRESGVPDRFTGSGSGTDFTLTISSVQAEDLAVYYCQNDYSYPYTFGGGTKLEIK

SEQ ID NO: 24 - protein, 5 aa, Artificial Sequence
  linker
GGGGS

SEQ ID NO: 25 - protein, 25 aa, Artificial Sequence
  linker
GGGGSGGGGSGASAAGGGGSGGGGS

SEQ ID NO: 26 - protein, 25 aa, Artificial Sequence
  linker
GGGGSGGGGSGGGGSGGGGSGGGGS

SEQ ID NO: 27 - protein, 250 aa, Artificial Sequence
  anti-CD123 scFv
EVQLQQSGPELVKPGASVKMSCKASGYTFTDYYMKWVKQSHGKSLEWIGDIIPSNGATFYNQKFKGKATLTVDRSSSTAYMHLNSLTSEDSAVYYCTRSHLLRASWFAYWGQGTLVTVSAASGGGGSGGGGSGGGGSDFVMTQSPSSLTVTAGEKVTMSCKSSQSLLNSGNQKNYLTWYLQKPGQPPKLLIYWASTRESGVPDRFTGSGSGTDFTLTISSVQAEDLAVYYCQNDYSYPYTFGGGTKLEIK

SEQ ID NO: 28 - protein, 10 aa, Homo sapiens
KPLPEVTDEY

SEQ ID NO: 29 - protein, 367 aa, Artificial Sequence
  humanized homo sapiens/mus musculus chimera
MRRMQLLLLIALSLALVTNSEFKPLPEVTDEYAAAGPGGGGSKILVKQSPMLVAYDNAVNLSCKYSYNLFSREFRASLHKGLDSAVEVCVVYGNYSQQLQVYSKTGFNCDGKLGNESVTFYLQNLYVNQTDIYFCKIEVMAPPPALDNEKSNGTIIHVKGKHLCPSPLFPGPSKPFWVLVVVGGVLACYSLLVTVAFIIFWVRSKRSRGGHSDYMNMTPRRPGPTRKHYQPYAPPRDFAAYRSGGGGSGGGASGGGGSFSRSADAPAYQQGQNQLYNELNLGRREEYDVLDKRRGRDPEMGGKPRRKNPQEGLYNELQKDKMAEAYSEIGMKGERRRGKGHDGLYQGLSTATKDTYGALHMQALPPR

SEQ ID NO: 30 - protein, 379 aa, Artificial Sequence
  humanized homo sapiens/mus musculus chimera
MRRMQLLLLIALSLALVTNSEFKPLPEVTDEYAAAGPGGGGSKILVKQSPMLVAYDNAVNLSCKYSYNLFSREFRASLHKGLDSAVEVCVVYGNYSQQLQVYSKTGFNCDGKLGNESVTFYLQNLYVNQTDIYFCKIEVMAPPPALDNEKSNGTIIHVKGKHLCPSPLFPGPSKPFWVLVVVGGVLACYSLLVTVAFIIFWVRSKRSRGGGGSKRGRKKLLYIFKQPFMRPVQTTQEEDGCSCRFPEEEEGGCELGGGGSGGGASGGGGSFSRSADAPAYQQGQNQLYNELNLGRREEYDVLDKRRGRDPEMGGKPRRKNPQEGLYNELQKDKMAEAYSEIGMKGERRRGKGHDGLYQGLSTATKDTYGALHMQALPPR

SEQ ID NO: 31 - DNA, 1101 bp, Artificial Sequence
  humanized homo sapiens/mus musculus chimera
atgcgccgcatgcagctgctgcttctgatcgctctgagcctggctcttgtgaccaactctgaattcaaacccctacctgaagtgactgatgagtatgctgccgctgggcccggaggaggcggcagcaagatcctggtcaaacagtcccctatgctggtcgcttacgacaacgccgttaatctgagttgcaaatatagttacaacctgtttagccgggaatttcgcgcatctctccacaagggactggattctgcggttgaggtttgtgtggtctatggcaattatagccagcaactgcaagtgtacagcaaaacaggctttaactgcgacgggaaactcgggaacgaatcagtgaccttctatctgcagaacctgtacgttaaccaaacagatatttacttctgcaagatagaggtgatggctccaccgccagcactggataacgagaagtccaatggaaccatcattcacgtcaaggggaagcatctgtgtccttccccgttgttccctgggccgagcaaacccttttgggtgcttgtggtagttggcggggtattggcctgctattcccttctcgtaactgtggccttcatcatcttctgggtcagatctaagaggtctaggggcgggcatagcgactacatgaacatgacacccaggcggcctggccccactcgcaaacactaccagccatacgcaccaccaagagactttgccgcatatcggagtggtggcggcgggtcaggaggtggagctagcggtggaggaggttccttctctaggtcagctgatgctcccgcctatcagcaaggtcagaaccagctctacaatgagctgaatctgggacgtcgggaggagtacgacgtgctggataaacgaagaggacgcgatcccgagatgggtgggaagcctaggcgcaagaatccccaggaaggcctctacaatgaactgcagaaagacaagatggccgaagcctacagcgagattggcatgaaaggggagcgacggagaggaaagggacatgacgggttgtatcagggtctttccactgcgacaaaggatacctatggggctctgcacatgcaagcactgccacctaga

SEQ ID NO: 32 - DNA, 1137 bp, Artificial Sequence
  humanized homo sapiens/mus musculus chimera
atgcgccgcatgcagctgctgcttctgatcgctctgagcctggctcttgtgaccaactctgaattcaaacccctacctgaagtgactgatgagtatgctgccgctgggcccggaggaggcggcagcaagatcctggtcaaacagtcccctatgctggtcgcttacgacaacgccgttaatctgagttgcaaatatagttacaacctgtttagccgggaatttcgcgcatctctccacaagggactggattctgcggttgaggtttgtgtggtctatggcaattatagccagcaactgcaagtgtacagcaaaacaggctttaactgcgacgggaaactcgggaacgaatcagtgaccttctatctgcagaacctgtacgttaaccaaacagatatttacttctgcaagatagaggtgatggctccaccgccagcactggataacgagaagtccaatggaaccatcattcacgtcaaggggaagcatctgtgtccttccccgttgttccctgggccgagcaaacccttttgggtgcttgtggtagttggcggggtattggcctgctattcccttctcgtaactgtggccttcatcatcttctgggtcagatctaagaggtctaggggcgggggcgggtcaaaacgcggacggaagaaactgctgtacatcttcaagcagcccttcatgcgccccgtgcagacaacacaggaagaggacggttgcagctgccgatttcccgaagaggaggagggaggctgtgaattgggtggcggcgggtcaggaggtggagctagcggtggaggaggttccttctctaggtcagctgatgctcccgcctatcagcaaggtcagaaccagctctacaatgagctgaatctgggacgtcgggaggagtacgacgtgctggataaacgaagaggacgcgatcccgagatgggtgggaagcctaggcgcaagaatccccaggaaggcctctacaatgaactgcagaaagacaagatggccgaagcctacagcgagattggcatgaaaggggagcgacggagaggaaagggacatgacgggttgtatcagggtctttccactgcgacaaaggatacctatggggctctgcacatgcaagcactgccacctaga